European Patent Specification EP 3 986 465 B1, published May 13, 2026. Title: Site-specific, kinetically inert conjugation of labels and/or carriers to target molecules such as His-tagged proteins via metal complex reagents. Applicant: Max-Planck-Gesellschaft zur Foerderung der Wissenschaften e.V. Universitaet Heidelberg. The sequence listing filed with the application follows.

SEQUENCE LISTING (16 sequences)

SEQ ID NO: 1 - protein, 6 aa, Artificial Sequence
  Consensus sequence chelating peptide
GHHPHG

SEQ ID NO: 2 - protein, 11 aa, Artificial Sequence
  Consensus sequence chelating peptide
GHHPHGHHPHG

SEQ ID NO: 3 - protein, 16 aa, Artificial Sequence
  Consensus sequence chelating peptide
GHHPHGHHPHGHHPHG

SEQ ID NO: 4 - protein, 20 aa, Artificial Sequence
  Metal cation ligand amino acid motif k=2
  VARIANT 1: X = G, A, F, W, M, Y, C, D, E, Q, H, K, P, S, T, N, R, U, O
  VARIANT 2..4: X = is absent or G, A, F, W, M, Y, C, D, E, Q, H, K, P, S, T, N, R, U, O
  VARIANT 5..10: X = is absent or L, I, V
  VARIANT 11: X = G, A, F, W, M, Y, C, D, E, Q, H, K, P, S, T, N, R, U, O
  VARIANT 12..14: X= absent or G, A, F, W, M, Y, C, D, E, Q, H, K, P, S, T, N, R, U, O
  VARIANT 15..20: X = absent or L, I, V
XXXXXXXXXXXXXXXXXXXX

SEQ ID NO: 5 - protein, 30 aa, Artificial Sequence
  Metal cation ligand amino acid motif k=3
  VARIANT 1: X = G, A, F, W, M, Y, C, D, E, Q, H, K, P, S, T, N, R, U, O
  VARIANT 2..4: X = absent or G, A, F, W, M, Y, C, D, E, Q, H, K, P, S, T, N, R, U, O
  VARIANT 5..10: X = absent or L, I, V
  VARIANT 11: X = G, A, F, W, M, Y, C, D, E, Q, H, K, P, S, T, N, R, U, O
  VARIANT 12..14: X = absent or G, A, F, W, M, Y, C, D, E, Q, H, K, P, S, T, N, R, U, O
  VARIANT 15..20: X = absent or L, I, V
  VARIANT 21: X = G, A, F, W, M, Y, C, D, E, Q, H, K, P, S, T, N, R, U, O
  VARIANT 22..24: X = absent or G, A, F, W, M, Y, C, D, E, Q, H, K, P, S, T, N, R, U, O
  VARIANT 25..30: X = absent or L, I, V
XXXXXXXXXXXXXXXXXXXXXXXXXXXXXX

SEQ ID NO: 6 - protein, 40 aa, Artificial Sequence
  Metal cation ligand amino acid motif k=4
  VARIANT 1: X = G, A, F, W, M, Y, C, D, E, Q, H, K, P, S, T, N, R, U, O
  VARIANT 2..4: X = absent or G, A, F, W, M, Y, C, D, E, Q, H, K, P, S, T, N, R, U, O
  VARIANT 5..10: X = absent or L, I, V
  VARIANT 11: X = G, A, F, W, M, Y, C, D, E, Q, H, K, P, S, T, N, R, U, O
  VARIANT 12..14: X = absent or G, A, F, W, M, Y, C, D, E, Q, H, K, P, S, T, N, R, U, O
  VARIANT 15..20: X = absent or L, I, V
  VARIANT 21: X = G, A, F, W, M, Y, C, D, E, Q, H, K, P, S, T, N, R, U, O
  VARIANT 22..24: X = absent or G, A, F, W, M, Y, C, D, E, Q, H, K, P, S, T, N, R, U, O
  VARIANT 25..30: X = absent or L, I, V
  VARIANT 31: X = G, A, F, W, M, Y, C, D, E, Q, H, K, P, S, T, N, R, U, O
  VARIANT 32..34: X = absent or G, A, F, W, M, Y, C, D, E, Q, H, K, P, S, T, N, R, U, O
  VARIANT 35..40: X = absent or L, I, V
XXXXXXXXXXXXXXXXXXXXXXXXXXXXXXXXXXXXXXXX

SEQ ID NO: 7 - protein, 50 aa, Artificial Sequence
  Metal cation ligand amino acid motif k=5
  VARIANT 1: X = G, A, F, W, M, Y, C, D, E, Q, H, K, P, S, T, N, R, U, O
  VARIANT 2..4: X = absent or G, A, F, W, M, Y, C, D, E, Q, H, K, P, S, T, N, R, U, O
  VARIANT 5..10: X = absent or L, I, V
  VARIANT 11: X = G, A, F, W, M, Y, C, D, E, Q, H, K, P, S, T, N, R, U, O
  VARIANT 12..14: X = absent or G, A, F, W, M, Y, C, D, E, Q, H, K, P, S, T, N, R, U, O
  VARIANT 15..20: X = absent or L, I, V
  VARIANT 21: X = G, A, F, W, M, Y, C, D, E, Q, H, K, P, S, T, N, R, U, O
  VARIANT 22..24: X = absent or G, A, F, W, M, Y, C, D, E, Q, H, K, P, S, T, N, R, U, O
  VARIANT 25..30: X = absent or L, I, V
  VARIANT 31: X = G, A, F, W, M, Y, C, D, E, Q, H, K, P, S, T, N, R, U, O
  VARIANT 32..34: X = absent or G, A, F, W, M, Y, C, D, E, Q, H, K, P, S, T, N, R, U, O
  VARIANT 35..40: X = absent or L, I, V
  VARIANT 41: X = G, A, F, W, M, Y, C, D, E, Q, H, K, P, S, T, N, R, U, O
  VARIANT 42..44: X = absent or G, A, F, W, M, Y, C, D, E, Q, H, K, P, S, T, N, R, U, O
  VARIANT 45..50: X is absent or L, I, V
XXXXXXXXXXXXXXXXXXXXXXXXXXXXXXXXXXXXXXXXXXXXXXXXXX

SEQ ID NO: 8 - protein, 60 aa, Artificial Sequence
  Metal cation ligand amino acid motif k=6
  VARIANT 1: X = G, A, F, W, M, Y, C, D, E, Q, H, K, P, S, T, N, R, U, O
  VARIANT 2..4: X = absent or G, A, F, W, M, Y, C, D, E, Q, H, K, P, S, T, N, R, U, O
  VARIANT 5..10: X = absent or L, I, V
  VARIANT 11: X = G, A, F, W, M, Y, C, D, E, Q, H, K, P, S, T, N, R, U, O
  VARIANT 12..14: X = absent or G, A, F, W, M, Y, C, D, E, Q, H, K, P, S, T, N, R, U, O
  VARIANT 15..20: X = absent or L, I, V
  VARIANT 21: X = G, A, F, W, M, Y, C, D, E, Q, H, K, P, S, T, N, R, U, O
  VARIANT 22..24: X = absent or G, A, F, W, M, Y, C, D, E, Q, H, K, P, S, T, N, R, U, O
  VARIANT 25..30: X = absent or L, I, V
  VARIANT 31: X = G, A, F, W, M, Y, C, D, E, Q, H, K, P, S, T, N, R, U, O
  VARIANT 32..34: X = absent or G, A, F, W, M, Y, C, D, E, Q, H, K, P, S, T, N, R, U, O
  VARIANT 35..40: X = absent or L, I, V
  VARIANT 41: X = G, A, F, W, M, Y, C, D, E, Q, H, K, P, S, T, N, R, U, O
  VARIANT 42..44: X = absent or G, A, F, W, M, Y, C, D, E, Q, H, K, P, S, T, N, R, U, O
  VARIANT 45..50: X = absent or L, I, V
  VARIANT 51: X = G, A, F, W, M, Y, C, D, E, Q, H, K, P, S, T, N, R, U, O
  VARIANT 52..54: X = absent or G, A, F, W, M, Y, C, D, E, Q, H, K, P, S, T, N, R, U, O
  VARIANT 55..60: X = absent or L, I, V
XXXXXXXXXXXXXXXXXXXXXXXXXXXXXXXXXXXXXXXXXXXXXXXXXXXXXXXXXXXX

SEQ ID NO: 9 - protein, 20 aa, Artificial Sequence
  Spaced histidine tag k=2
  VARIANT 2..4: X = absent or H
  VARIANT 5..10: X = absent or G, A, F, W, M, Y, C, D, E, Q, H, K, P, S, T, N, R, L, I, V, U, O
  VARIANT 12..14: X = absent or H
  VARIANT 15..20: X = absent or G, A, F, W, M, Y, C, D, E, Q, H, K, P, S, T, N, R, L, I, V, U, O
HXXXXXXXXXHXXXXXXXXX

SEQ ID NO: 10 - protein, 30 aa, Artificial Sequence
  Spaced histidine tag k=3
  VARIANT 2..4: X = absent or H
  VARIANT 5..10: X = absent or G, A, F, W, M, Y, C, D, E, Q, H, K, P, S, T, N, R, L, I, V, U, O
  VARIANT 12..14: X = absent or H
  VARIANT 15..20: X = absent or G, A, F, W, M, Y, C, D, E, Q, H, K, P, S, T, N, R, L, I, V, U, O
  VARIANT 22..24: X = absent or H
  VARIANT 25..30: X = absent or G, A, F, W, M, Y, C, D, E, Q, H, K, P, S, T, N, R, L, I, V, U, O
HXXXXXXXXXHXXXXXXXXXHXXXXXXXXX

SEQ ID NO: 11 - protein, 40 aa, Artificial Sequence
  Spaced histidine tag k=4
  VARIANT 2..4: X = absent or H
  VARIANT 5..10: X = absent or G, A, F, W, M, Y, C, D, E, Q, H, K, P, S, T, N, R, L, I, V, U, O
  VARIANT 12..14: X = absent or H
  VARIANT 15..20: X = absent or G, A, F, W, M, Y, C, D, E, Q, H, K, P, S, T, N, R, L, I, V, U, O
  VARIANT 22..24: X = absent or H
  VARIANT 25..30: X = absent or G, A, F, W, M, Y, C, D, E, Q, H, K, P, S, T, N, R, L, I, V, U, O
  VARIANT 32..34: X = absent or H
  VARIANT 35..40: X = absent or G, A, F, W, M, Y, C, D, E, Q, H, K, P, S, T, N, R, L, I, V, U, O
HXXXXXXXXXHXXXXXXXXXHXXXXXXXXXHXXXXXXXXX

SEQ ID NO: 12 - protein, 50 aa, Artificial Sequence
  Spaced histidine tag k=5
  VARIANT 2..4: X = absent or H
  VARIANT 5..10: X = absent or G, A, F, W, M, Y, C, D, E, Q, H, K, P, S, T, N, R, L, I, V, U, O
  VARIANT 12..14: X = absent or H
  VARIANT 15..20: X = absent or G, A, F, W, M, Y, C, D, E, Q, H, K, P, S, T, N, R, L, I, V, U, O
  VARIANT 22..24: X = absent or H
  VARIANT 25..30: X = absent or G, A, F, W, M, Y, C, D, E, Q, H, K, P, S, T, N, R, L, I, V, U, O
  VARIANT 32..34: X = absent or H
  VARIANT 35..40: X = absent or G, A, F, W, M, Y, C, D, E, Q, H, K, P, S, T, N, R, L, I, V, U, O
  VARIANT 42..44: X = absent or H
  VARIANT 45..50: X = absent or G, A, F, W, M, Y, C, D, E, Q, H, K, P, S, T, N, R, L, I, V, U, O
HXXXXXXXXXHXXXXXXXXXHXXXXXXXXXHXXXXXXXXXHXXXXXXXXX

SEQ ID NO: 13 - protein, 60 aa, Artificial Sequence
  Spaced histidine tag k=6
  VARIANT 2..4: X = absent or H
  VARIANT 5..10: X = absent or G, A, F, W, M, Y, C, D, E, Q, H, K, P, S, T, N, R, L, I, V, U, O
  VARIANT 12..14: X = absent or H
  VARIANT 15..20: X = absent or G, A, F, W, M, Y, C, D, E, Q, H, K, P, S, T, N, R, L, I, V, U, O
  VARIANT 22..24: X = absent or H
  VARIANT 25..30: X = absent or G, A, F, W, M, Y, C, D, E, Q, H, K, P, S, T, N, R, L, I, V, U, O
  VARIANT 32..34: X = absent or H
  VARIANT 35..40: X = absent or G, A, F, W, M, Y, C, D, E, Q, H, K, P, S, T, N, R, L, I, V, U, O
  VARIANT 42..44: X = absent or H
  VARIANT 45..50: X = absent or G, A, F, W, M, Y, C, D, E, Q, H, K, P, S, T, N, R, L, I, V, U, O
  VARIANT 52..54: X = absent or H
  VARIANT 55..60: X = absent or G, A, F, W, M, Y, C, D, E, Q, H, K, P, S, T, N, R, L, I, V, U, O
HXXXXXXXXXHXXXXXXXXXHXXXXXXXXXHXXXXXXXXXHXXXXXXXXXHXXXXXXXXX

SEQ ID NO: 14 - protein, 266 aa, Artificial Sequence
  His-GFP
MGSSHHHHHHGSSVSKGEELFTGVVPILVELDGDVNGHKFSVRGEGEGDATNGKLTLKFICTTGKLPVPWPTLVTTLTYGVQCFSRYPDHMKQHDFFKSAMPEGYVQERTISFKDDGTYKTRAEVKFEGDTLVNRIELKGIDFKEDGNILGHKLEYNFNSHNVYITADKQKNGIKANFKIRHNVEDGSVQLADHYQQNTPIGDGPVLLPDNHYLSTQSKLSKDPNEKRDHMVLLEFVTAAGITLGMDELYKGIEENLYFQSNIGSG

SEQ ID NO: 15 - protein, 591 aa, Artificial Sequence
  His-PercevalHR
MKHHHHHHHGASMKKVESIIRPEKLEIVKKALSDAGYVGMTVSEVKGSGVQGGIFERYRGRVYSAGYNSDNVYITADKQKNGIKANFKIRHNIEDGGVQLADHYQQNTPIGDGPVLLPDNHYLSFQSKLSKDPNEKRDHMVLLEFVTAAGITLGMDELYKGGSGGMVSKGEELFTGVVPILVELDGDVNGHKFSVSGEGEGDATYGKLTLKLICTTGKLPVPWPTLVTTLGYGLQCFARYPDHMKQHDFFKSAMPEGYVQERTIFFKDDGNYKTRAEVKFEGDTLVNRIELKGIDFKEDGNILGHKLEYNGTIVDLIPKVKIELVVKEEDVDNVIDIICENARTGNPGDGKIFVIPVERVVRVRTKEEGASGGGSGGGGASGMKKVEAIIRPEKLEIVKKALSDAGYVGMTVSEVKGRGAGGGDLIPKVKIELVVKEEDVDNVIDIICENARTGNPGDGKIFVIPVERIVRVRTKEEGASGGGGGSGGASGMKKVEAIIRPEKLEIVKKALNDDGYVGMTVSEVKGRGAGGGDLIPKVKIELVVKEEDVDNIIDIICENARTGNPGDGKIFVIPVERVVRPRTKEEGKEAL

SEQ ID NO: 16 - protein, 156 aa, Artificial Sequence
  enzyme Sortase A
MQAKPQIPKDKSKVAGYIEIPDADIKEPVYPGPATREQLNRGVSFAEENESLDDQNISIAGHTFIDRPNYQFTNLKAAKKGSMVYFKVGNETRKYKMTSIRNVKPTAVEVLDEQKGKDKQLTLITCDDYNEETGVWETRKIFVATEVKLEHHHHHH